European Patent Specification EP 3 827 846 B1, published October 2, 2024. Title: COMPOSITIONS, COMBINATIONS AND RELATED METHODS FOR PHOTOIMMUNOTHERAPY. Applicant: Rakuten Medical, Inc. The sequence listing filed with the application follows.

SEQUENCE LISTING (52 sequences)

SEQ ID NO: 1 - protein, 9 aa, Artificial Sequence
  homing peptide
CRGDKGPDC

SEQ ID NO: 2 - protein, 10 aa, Artificial Sequence
  homing peptide
CCRGDKGPDC

SEQ ID NO: 3 - protein, 16 aa, Artificial Sequence
  homing peptide
AKPAPPKPEPKPKKAP

SEQ ID NO: 4 - protein, 15 aa, Artificial Sequence
  homing peptide
AKVKDEPQRRSARLS

SEQ ID NO: 5 - protein, 7 aa, Artificial Sequence
  homing peptide
CAGALCY

SEQ ID NO: 6 - protein, 9 aa, Artificial Sequence
  homing peptide
CAGRRSAYC

SEQ ID NO: 7 - protein, 9 aa, Artificial Sequence
  homing peptide
CARSKNKDC

SEQ ID NO: 8 - protein, 9 aa, Artificial Sequence
  homing peptide
CDCRGDCFC

SEQ ID NO: 9 - protein, 5 aa, Artificial Sequence
  homing peptide
CDTRL

SEQ ID NO: 10 - protein, 5 aa, Artificial Sequence
  homing peptide
CGKRK

SEQ ID NO: 11 - protein, 10 aa, Artificial Sequence
  homing peptide
CGLIIQKNEC

SEQ ID NO: 12 - protein, 7 aa, Artificial Sequence
  homing peptide
CGNKRTR

SEQ ID NO: 13 - protein, 9 aa, Artificial Sequence
  homing peptide
CGNKRTRGC

SEQ ID NO: 14 - protein, 9 aa, Artificial Sequence
  homing peptide
CGRRAGGSC

SEQ ID NO: 15 - protein, 7 aa, Artificial Sequence
  homing peptide
CKAAKNK

SEQ ID NO: 16 - protein, 11 aa, Artificial Sequence
  homing peptide
CKGGRAKDCGG

SEQ ID NO: 17 - protein, 9 aa, Artificial Sequence
  homing peptide
CLSDGKRKC

SEQ ID NO: 18 - protein, 12 aa, Artificial Sequence
  homing peptide
CMYIEALDKYAC

SEQ ID NO: 19 - protein, 12 aa, Artificial Sequence
  homing peptide
KKCGGGGIRLRG

SEQ ID NO: 20 - protein, 10 aa, Artificial Sequence
  homing peptide
CNAGESSKNC

SEQ ID NO: 21 - protein, 5 aa, Artificial Sequence
  homing peptide
CNGRC

SEQ ID NO: 22 - protein, 9 aa, Artificial Sequence
  homing peptide
CNRRTKAGC

SEQ ID NO: 23 - protein, 9 aa, Artificial Sequence
  homing peptide
CPGPEGAGC

SEQ ID NO: 24 - protein, 9 aa, Artificial Sequence
  homing peptide
CPKTRRPVC

SEQ ID NO: 25 - protein, 9 aa, Artificial Sequence
  homing peptide
CPRECESIC

SEQ ID NO: 26 - protein, 9 aa, Artificial Sequence
  homing peptide
CRAKSKVAC

SEQ ID NO: 27 - protein, 9 aa, Artificial Sequence
  homing peptide
CREAGRKAC

SEQ ID NO: 28 - protein, 5 aa, Artificial Sequence
  homing peptide
CREKA

SEQ ID NO: 29 - protein, 9 aa, Artificial Sequence
  homing peptide
CRGDKGPDC

SEQ ID NO: 30 - protein, 7 aa, Artificial Sequence
  homing peptide
CRGRRST

SEQ ID NO: 31 - protein, 6 aa, Artificial Sequence
  homing peptide
CRKDKC

SEQ ID NO: 32 - protein, 5 aa, Artificial Sequence
  homing peptide
CRPPR

SEQ ID NO: 33 - protein, 9 aa, Artificial Sequence
  homing peptide
CRRETAWAC

SEQ ID NO: 34 - protein, 6 aa, Artificial Sequence
  homing peptide
CRSRKG

SEQ ID NO: 35 - protein, 9 aa, Artificial Sequence
  homing peptide
CSRPRRSEC

SEQ ID NO: 36 - protein, 10 aa, Artificial Sequence
  homing peptide
CTTHWGFTLC

SEQ ID NO: 37 - protein, 9 aa, Artificial Sequence
  homing peptide
CVPELGHEC

SEQ ID NO: 38 - protein, 13 aa, Artificial Sequence
  homing peptide
EKGEGALPTGKSK

SEQ ID NO: 39 - protein, 6 aa, Artificial Sequence
  homing peptide
FALGEA

SEQ ID NO: 40 - protein, 13 aa, Artificial Sequence
  homing peptide
GLNGLSSADPSSD

SEQ ID NO: 41 - protein, 8 aa, Artificial Sequence
  homing peptide
GSMSIARL

SEQ ID NO: 42 - protein, 8 aa, Artificial Sequence
  homing peptide
GVSFLEYR

SEQ ID NO: 43 - protein, 7 aa, Artificial Sequence
  homing peptide
IFLLWQR

SEQ ID NO: 44 - protein, 10 aa, Artificial Sequence
  homing peptide
IFLLWQRCRR

SEQ ID NO: 45 - protein, 5 aa, Artificial Sequence
  homing peptide
PEPHC

SEQ ID NO: 46 - protein, 13 aa, Artificial Sequence
  homing peptide
PISNDQKVSDDDK

SEQ ID NO: 47 - protein, 15 aa, Artificial Sequence
  homing peptide
RMWPSSTVNLSAGRR

SEQ ID NO: 48 - protein, 7 aa, Artificial Sequence
  homing peptide
RPARPAR

SEQ ID NO: 49 - protein, 7 aa, Artificial Sequence
  homing peptide
SMSIARL

SEQ ID NO: 50 - protein, 13 aa, Artificial Sequence
  homing peptide
VDEDRASLLKSQE

SEQ ID NO: 51 - protein, 7 aa, Artificial Sequence
  homing peptide
VSFLEYR

SEQ ID NO: 52 - protein, 11 aa, Artificial Sequence
  homing peptide
WNAPAEEWGNW